European Patent Application EP 4 194 466 A1, published June 14, 2023. Title: ANTIVIRAL COMPOSITION FOR CORONAVIRUS. Applicant: Novelgen. The sequence listing filed with the application follows.

SEQUENCE LISTING (28 sequences)

SEQ ID NO: 1 - protein, 10 aa, Artificial Sequence
  VH CDR1
GYTFTSYVMH

SEQ ID NO: 2 - protein, 7 aa, Artificial Sequence
  VH CDR2
INPYNDG

SEQ ID NO: 3 - protein, 11 aa, Artificial Sequence
  VH CDR3
GAYKRGYAMDY

SEQ ID NO: 4 - protein, 17 aa, Artificial Sequence
  VL CDR1
KSSQSLFNSRTRKNYLA

SEQ ID NO: 5 - protein, 7 aa, Artificial Sequence
  VL CDR2
WASTRES

SEQ ID NO: 6 - protein, 9 aa, Artificial Sequence
  VL CDR3
KQSYYHMYT

SEQ ID NO: 7 - protein, 121 aa, Artificial Sequence
  VH
EVQLQQSGPELVKPGASVKMSCKASGYTFTSYVMHWVKQKPGQGLEWIGYINPYNDGTKYNEKFKGKATLTSDKSSSTAYMELSSLTSEDSAVYYCARGAYKRGYAMDYWGQGTSVTVSSR

SEQ ID NO: 8 - protein, 113 aa, Artificial Sequence
  VL
DLVMSQSPSSLAVSAGEKVTMSCKSSQSLFNSRTRKNYLAWYQQKPGQSPKLLIYWASTRESGVPDRFTGSGSGTDFTLTISSVQAEDLAVYYCKQSYYHMYTFGSGTKLEIK

SEQ ID NO: 9 - protein, 249 aa, Artificial Sequence
  NVG308(scFv)
EVQLQQSGPELVKPGASVKMSCKASGYTFTSYVMHWVKQKPGQGLEWIGYINPYNDGTKYNEKFKGKATLTSDKSSSTAYMELSSLTSEDSAVYYCARGAYKRGYAMDYWGQGTSVTVSSRGGGGSGGGGSGGGGSDLVMSQSPSSLAVSAGEKVTMSCKSSQSLFNSRTRKNYLAWYQQKPGQSPKLLIYWASTRESGVPDRFTGSGSGTDFTLTISSVQAEDLAVYYCKQSYYHMYTFGSGTKLEIK

SEQ ID NO: 10 - DNA, 747 bp, Artificial Sequence
  NVG308 gene
gaggtccagctgcagcagtctggacctgagctggtaaagcctggggcttcagtgaagatgtcctgcaaggcttctggatacacattcactagctatgttatgcactgggtgaagcagaagcctgggcagggccttgagtggattggatatattaatccttacaatgatggtactaagtacaatgagaagttcaaaggcaaggccacactgacttcagacaaatcctccagcacagcctacatggagctcagcagcctgacctctgaggactctgcggtctattactgtgcaagaggggcctataaaaggggatatgctatggactactggggtcaaggaacctcagtcaccgtctcctctagaggtgggggcggttcgggtggcgggggctcgggcgggggtggctcagatcttgtgatgtcacagtctccatcctccctggctgtgtcagcaggagagaaggtcactatgagctgcaaatccagtcagagtctgttcaacagtagaacccgaaagaactacttggcttggtaccagcagaaaccagggcagtctcctaaactgctgatctactgggcatccactagggaatctggggtccctgatcgcttcacaggcagtggatctgggacagatttcactctcaccatcagcagtgtgcaggctgaagacctggcagtttattactgcaagcaatcttattatcacatgtatacgttcggatcggggaccaagctggaaataaaa

SEQ ID NO: 11 - DNA, 20 bp, Artificial Sequence
  PEDV_forward primer
tgtctctgcgtcttttggtg

SEQ ID NO: 12 - DNA, 20 bp, Artificial Sequence
  PEDV_reverse primer
ctgccacttgcaggatcata

SEQ ID NO: 13 - DNA, 20 bp, Artificial Sequence
  SARS-CoV-2_forward primer
cagatgctggcttcatcaaa

SEQ ID NO: 14 - DNA, 20 bp, Artificial Sequence
  SARS-CoV-2_reverse primer
cattgaggcggtcaatttct

SEQ ID NO: 15 - DNA, 21 bp, Artificial Sequence
  hCoV-OC43 Spike surface glycoprotein_forward primer
agctatacccaatggcaggaa

SEQ ID NO: 16 - DNA, 19 bp, Artificial Sequence
  hCoV-OC43 Spike surface glycoprotein_reverse primer
ccagtggtaatcgctccac

SEQ ID NO: 17 - DNA, 22 bp, Artificial Sequence
  hCoV-OC43 Hemagglutinin-esterase_forward primer
cgcatgtaaatggagattggtt

SEQ ID NO: 18 - DNA, 22 bp, Artificial Sequence
  hCoV-OC43 Hemagglutinin-esterase_reverse primer
cccaaaagaatgccaagcaaaa

SEQ ID NO: 19 - DNA, 22 bp, Artificial Sequence
  SARS-CoV-2_RdRP gene_forward primer
gtgaratggtcatgtgtggcgg

SEQ ID NO: 20 - DNA, 26 bp, Artificial Sequence
  SARS-CoV-2_RdRP gene_reverse primer
caratgttaaasacactattagcata

SEQ ID NO: 21 - DNA, 26 bp, Artificial Sequence
  SARS-CoV-2_E gene_forward primer
acaggtacgttaatagttaatagcgt

SEQ ID NO: 22 - DNA, 22 bp, Artificial Sequence
  SARS-CoV-2_E gene_reverse primer
atattgcagcagtacgcacaca

SEQ ID NO: 23 - DNA, 19 bp, Artificial Sequence
  SARS-CoV-2_N gene_forward primer
cacattggcacccgcaatc

SEQ ID NO: 24 - DNA, 20 bp, Artificial Sequence
  SARS-CoV-2_N gene_reverse primer
caggaacgagaagaggcttg

SEQ ID NO: 25 - DNA, 29 bp, Artificial Sequence
  hCoV-OC43_N gene_forward primer
agtactgctatttcttgttcaaacatgtg

SEQ ID NO: 26 - DNA, 26 bp, Artificial Sequence
  hCoV-OC43_N gene_reverse primer
gctctacgacttcgtctgtttttaga

SEQ ID NO: 27 - DNA, 17 bp, Artificial Sequence
  PEDV_N gene_forward primer
gatcgtggccgcaaacg

SEQ ID NO: 28 - DNA, 18 bp, Artificial Sequence
  PEDV_N gene_reverse primer
tgccattgccacgactcc